European Patent Application EP 4 219 705 A1, published August 2, 2023. Title: Novel Recombinant Factor C and Method for Producing the Same, and Method for Measuring Endotoxin. Applicant: SEIKAGAKU CORPORATION. Application EP. The sequence listing filed with the application follows.

SEQUENCE LISTING (10 sequences)

SEQ ID NO: 1 - DNA, 3060 bp, Tachypleus tridentatus
  source 1..3060: mol_type = genomic DNA
atggtcttagcgtcgtttttggtgtctggtttagttctagggatactagcccaacaaatgcgtccagttcagtccagaggagtagatctgggcttgtgtgatgaaacgaggttcgagtgtaagtgtggagatccaggctatgtgttcaacgtccctatgaaacaatgcacgtacttctatcgatggaggccttattgtaaaccatgtgatgacctggaggctaaggacatttgtccaaagtacaaacgatgtcaagagtgtaaggctggtcttgatagttgtgttacttgtccacctaacaaatatggtacttggtgtagcggtgaatgtcaatgtaagaatggaggtatctgtgaccagaggacaggagcttgtacctgtcgtgacagatatgaaggagcgcactgtgaaattctcaaaggttgtcctcttcttccatcggattctcaagttcaggaagtcagaaacccaccagataatccccaaactattgactacagctgttcaccagggttcaagcttaaaggcgtggcacgaattagctgtctcccaaatggacagtggagtagctttccacccaaatgtattcgagaatgtgccaaggtttcatctccagaacacgggaaagtgaatgctcctagtggcaatatgatagaaggggctactttacggttctcatgtgatagtccctactacttgattggtcaagaaacattaacctgccagggtaatggtcagtggagtggacaaataccacaatgtaagaagttggtcttctgtcctgaccttgatcctgtaaaccatgctgaacaccaggttaaaattggtgtggaacaaaaatatggtcagtttcctcaaggcactgaagtgacctatacgtgttcgggtaactacttcttgatgggttttaacaccttaaaatgtaaccctgatgggtcctggtcaggatcacagccatcctgtgttaaagtggcagacagagaggtcgactgtgacagtaaagctgtagacttcttggatgatgttggtgaacctgtcaggatccactgtcctgctggctgttctttgacagctggtactgtgtggggtacagccatataccacgaactttcctcagtgtgtcgtgcagccatccatgctggcaagcttccaaactctggaggggcggtgcatgtagtgaacaatggcccctactcggactttctgggtagtgacctgaatgggataaaatcggaagagttgaagtctcttgcccgcagttttcgatttgattatgtcagttcatccacagcaggtagatcaggatgtcctgatggatggtttgaggtagaagagaactgtgtgtacgttacatcaaaacagagagcctgggaaagagctcaaggtgtgtgtaccaatatggctgctcgtcttgctgtgctagacaaagatctaattccgagttccttgactgagactctacgagggaaagggttaacaaccacatggataggattgcacagactagatgctgagaagccctttgtttgggagctaatggatcgtagtaatgtggttctgaatgataacctaacattctgggcctctggcgaacctggaaatgaaactaactgtgtatatctggacatccgagatcagctgcagcctgtgtggaaaaccaagtcatgttttcagccctcaagctttgcttgcatgatggatttgtcagacagaaataaagccaaatgcgatgaccctggaccactggaaaatggacacgccacacttcatggacaaagtattgatgggttctatgctggttcttctataaggtacagctgtgaggttctccactacctcagtggaactgagaccgtaacttgtacaacaaatggcacatggagtgctcctaaacctcgatgtatcaaagtcatcacctgccaaaaccctcctgtaccatcatatggttctgtggaaatcaaacccccaagtcggacaaactcgatcagtcgtgttgggtcacctttcttgaggttgccacggttacccctcccattagccagagcagccaaacctcctccaaaacctagatcctcacaaccctctactgtggacttggcttctaaagttaaactacctgaaggtcattaccgggtagggtctcgagccatttacacgtgcgagtcgagatactacgaactacttggatctcaaggcagaagatgtgactctaatggaaactggagtggtcggcccgctagctgtattccagtttgtggacggtcagactctcctcgttctcctttcatctggaatgggaattctacagaaataggtcagtggccgtggcaggcaggaatctctcgatggcttgcagaccacaatatgtggtttctccagtgtggaggatccctattgaatgagaaatggatcgtcactgctgcccactgtgtcacctactctgctactgctgagataattgatcccagtcagtttaaaatctatctgggcaagtactaccgtgatgacagtagagacgatgactacgtacaagtaagagaggctctcgagatccacgtaaatcctaactacgaccccggcaatctcaactttgacatagccctaattcaactgaaaactcctgttactttgacaacacgagtccaaccaatctgtctgcctactgacatcacaacaagagaacacttgaaggagggaacattagcagtggtgacaggttggggtttgaatgaaaacaacacatattcagagatgattcaacaagctgtgctacctgttgttgcagcaagcacctgtgaagaggggtacaaggaagcagacttaccactgacagtaacagagaacatgttctgtgcaggttacaagaagggacgttatgatgcctgcagtggggacagtggaggaccattagtgtttgctgatgattcccgtaccgaaaggcggtgggtcttggaagggattgtcagctggggcagtcccagtggatgtggcaaggctaaccagtatgggggcttcactaaagttaacgtttttctatcatggattaggcagttcatttga

SEQ ID NO: 2 - protein, 1019 aa, Tachypleus tridentatus
MVLASFLVSGLVLGILAQQMRPVQSRGVDLGLCDETRFECKCGDPGYVFNVPMKQCTYFYRWRPYCKPCDDLEAKDICPKYKRCQECKAGLDSCVTCPPNKYGTWCSGECQCKNGGICDQRTGACTCRDRYEGAHCEILKGCPLLPSDSQVQEVRNPPDNPQTIDYSCSPGFKLKGVARISCLPNGQWSSFPPKCIRECAKVSSPEHGKVNAPSGNMIEGATLRFSCDSPYYLIGQETLTCQGNGQWSGQIPQCKKLVFCPDLDPVNHAEHQVKIGVEQKYGQFPQGTEVTYTCSGNYFLMGFNTLKCNPDGSWSGSQPSCVKVADREVDCDSKAVDFLDDVGEPVRIHCPAGCSLTAGTVWGTAIYHELSSVCRAAIHAGKLPNSGGAVHVVNNGPYSDFLGSDLNGIKSEELKSLARSFRFDYVSSSTAGRSGCPDGWFEVEENCVYVTSKQRAWERAQGVCTNMAARLAVLDKDLIPSSLTETLRGKGLTTTWIGLHRLDAEKPFVWELMDRSNVVLNDNLTFWASGEPGNETNCVYLDIRDQLQPVWKTKSCFQPSSFACMMDLSDRNKAKCDDPGPLENGHATLHGQSIDGFYAGSSIRYSCEVLHYLSGTETVTCTTNGTWSAPKPRCIKVITCQNPPVPSYGSVEIKPPSRTNSISRVGSPFLRLPRLPLPLARAAKPPPKPRSSQPSTVDLASKVKLPEGHYRVGSRAIYTCESRYYELLGSQGRRCDSNGNWSGRPASCIPVCGRSDSPRSPFIWNGNSTEIGQWPWQAGISRWLADHNMWFLQCGGSLLNEKWIVTAAHCVTYSATAEIIDPSQFKIYLGKYYRDDSRDDDYVQVREALEIHVNPNYDPGNLNFDIALIQLKTPVTLTTRVQPICLPTDITTREHLKEGTLAVVTGWGLNENNTYSEMIQQAVLPVVAASTCEEGYKEADLPLTVTENMFCAGYKKGRYDACSGDSGGPLVFADDSRTERRWVLEGIVSWGSPSGCGKANQYGGFTKVNVFLSWIRQFI

SEQ ID NO: 3 - DNA, 3060 bp, Carcinoscorpius rotundicauda
  source 1..3060: mol_type = genomic DNA
atggtcttagcgtcgtttttggtgtctggtttagttctagggctactagcccaaaaaatgcgcccagttcagtccaaaggagtagatctaggcttgtgtgatgaaacgaggttcgagtgtaagtgtggcgatccaggctatgtgttcaacattccagtgaaacaatgtacatacttttatcgatggaggccgtattgtaaaccatgtgatgacctggaggctaaggatatttgtccaaagtacaaacgatgtcaagagtgtaaggctggtcttgatagttgtgttacttgtccacctaacaaatatggtacttggtgtagcggtgaatgtcagtgtaagaatggaggtatctgtgaccagaggacaggagcttgtgcatgtcgtgacagatatgaaggggtgcactgtgaaattctcaaaggttgtcctcttcttccatcggattctcaggttcaggaagtcagaaatccaccagataatccccaaactattgactacagctgttcaccagggttcaagcttaagggtatggcacgaattagctgtctcccaaatggacagtggagtaactttccacccaaatgtattcgagaatgtgccatggtttcatctccagaacatgggaaagtgaatgctcttagtggtgatatgatagaaggggctactttacggttctcatgtgatagtccctactacttgattggtcaagaaacattaacctgtcagggtaatggtcagtggaatggacagataccacaatgtaagaacttggtcttctgtcctgacctggatcctgtaaaccatgctgaacacaaggttaaaattggtgtggaacaaaaatatggtcagtttcctcaaggcactgaagtgacctatacgtgttcgggtaactacttcttgatgggttttgacaccttaaaatgtaaccctgatgggtcttggtcaggatcacagccatcctgtgttaaagtggcagacagagaggtcgactgtgacagtaaagctgtagacttcttggatgatgttggtgaacctgtcaggatccactgtcctgctggctgttctttgacagctggtactgtgtggggtacagccatataccatgaactttcctcagtgtgtcgtgcagccatccatgctggcaagcttccaaactctggaggagcggtgcatgttgtgaacaatggcccctactcggactttctgggtagtgacctgaatgggataaaatcggaagagttgaagtctcttgcccggagtttccgattcgattatgtccgttcctccacagcaggtaaatcaggatgtcctgatggatggtttgaggtagacgagaactgtgtgtacgttacatcaaaacagagagcctgggaaagagctcaaggtgtgtgtaccaatatggctgctcgtcttgctgtgctggacaaagatgtaattccaaattcgttgactgagactctacgagggaaagggttaacaaccacgtggataggattgcacagactagatgctgagaagccctttatttgggagttaatggatcgtagtaatgtggttctgaatgataacctaacattctgggcctctggcgaacctggaaatgaaactaactgtgtatatatggacatccaagatcagttgcagtctgtgtggaaaaccaagtcatgttttcagccctcaagttttgcttgcatgatggatctgtcagacagaaataaagccaaatgcgatgatcctggatcactggaaaatggacacgccacacttcatggacaaagtattgatgggttctatgctggttcttctataaggtacagctgtgaggttctccactacctcagtggaactgaaaccgtaacttgtacaacaaatggcacatggagtgctcctaaacctcgatgtatcaaagtcatcacctgccaaaacccccctgtaccatcatatggttctgtggaaatcaaacccccaagtcggacaaactcgataagtcgtgttgggtcacctttcttgaggttgccacggttacccctcccattagctagagcagccaaacctcctccaaaacctagatcctcacaaccctctactgtggacttggcttctaaagttaaactacctgaaggtcattaccgggtagggtctcgagccatctacacgtgcgagtcgagatactacgaactacttggatctcaaggcagaagatgtgactctaatggaaactggagtggtcggccagcgagctgtattccagtttgtggacggtcagactctcctcgttctccttttatctggaatgggaattctacagaaataggtcagtggccgtggcaggcaggaatctctagatggcttgcagaccacaatatgtggtttctccagtgtggaggatctctattgaatgagaaatggatcgtcactgctgcccactgtgtcacctactctgctactgctgagattattgaccccaatcagtttaaaatgtatctgggcaagtactaccgtgatgacagtagagacgatgactatgtacaagtaagagaggctcttgagatccacgtgaatcctaactacgaccccggcaatctcaactttgacatagccctaattcaactgaaaactcctgttactttgacaacacgagtccaaccaatctgtctgcctactgacatcacaacaagagaacacttgaaggagggaacattagcagtggtgacaggttggggtttgaatgaaaacaacacctattcagagacgattcaacaagctgtgctacctgttgttgcagccagcacctgtgaagaggggtacaaggaagcagacttaccactgacagtaacagagaacatgttctgtgcaggttacaagaagggacgttatgatgcctgcagtggggacagtggaggacctttagtgtttgctgatgattcccgtaccgaaaggcggtgggtcttggaagggattgtcagctggggcagtcccagtggatgtggcaaggcgaaccagtacgggggcttcactaaagttaacgttttcctgtcatggattaggcagttcatttga

SEQ ID NO: 4 - protein, 1019 aa, Carcinoscorpius rotundicauda
MVLASFLVSGLVLGLLAQKMRPVQSKGVDLGLCDETRFECKCGDPGYVFNIPVKQCTYFYRWRPYCKPCDDLEAKDICPKYKRCQECKAGLDSCVTCPPNKYGTWCSGECQCKNGGICDQRTGACACRDRYEGVHCEILKGCPLLPSDSQVQEVRNPPDNPQTIDYSCSPGFKLKGMARISCLPNGQWSNFPPKCIRECAMVSSPEHGKVNALSGDMIEGATLRFSCDSPYYLIGQETLTCQGNGQWNGQIPQCKNLVFCPDLDPVNHAEHKVKIGVEQKYGQFPQGTEVTYTCSGNYFLMGFDTLKCNPDGSWSGSQPSCVKVADREVDCDSKAVDFLDDVGEPVRIHCPAGCSLTAGTVWGTAIYHELSSVCRAAIHAGKLPNSGGAVHVVNNGPYSDFLGSDLNGIKSEELKSLARSFRFDYVRSSTAGKSGCPDGWFEVDENCVYVTSKQRAWERAQGVCTNMAARLAVLDKDVIPNSLTETLRGKGLTTTWIGLHRLDAEKPFIWELMDRSNVVLNDNLTFWASGEPGNETNCVYMDIQDQLQSVWKTKSCFQPSSFACMMDLSDRNKAKCDDPGSLENGHATLHGQSIDGFYAGSSIRYSCEVLHYLSGTETVTCTTNGTWSAPKPRCIKVITCQNPPVPSYGSVEIKPPSRTNSISRVGSPFLRLPRLPLPLARAAKPPPKPRSSQPSTVDLASKVKLPEGHYRVGSRAIYTCESRYYELLGSQGRRCDSNGNWSGRPASCIPVCGRSDSPRSPFIWNGNSTEIGQWPWQAGISRWLADHNMWFLQCGGSLLNEKWIVTAAHCVTYSATAEIIDPNQFKMYLGKYYRDDSRDDDYVQVREALEIHVNPNYDPGNLNFDIALIQLKTPVTLTTRVQPICLPTDITTREHLKEGTLAVVTGWGLNENNTYSETIQQAVLPVVAASTCEEGYKEADLPLTVTENMFCAGYKKGRYDACSGDSGGPLVFADDSRTERRWVLEGIVSWGSPSGCGKANQYGGFTKVNVFLSWIRQFI

SEQ ID NO: 5 - DNA, 1203 bp, Tachypleus tridentatus
  source 1..1203: mol_type = genomic DNA
atgacgtggatatgtgtgataacgttgtttgctctggcttctgctacgttgggtaacaaagttagtagagtgggggtcctcttccccaagacacggaacgacaatgagtgtacagcaagagggggattgaaaggatcctgcaaatccctcatagactgtcctagtgtcttggctacgttgaaggacagttttcctgtcgtttgctcttggaatggtcgatttcagcctattgtctgctgtcctgatgcaatagcaccaccacctgtaaccacaacagctgtaactgtaatatctacaaaagaaccaaagcttccaagattacatatatcaggttgtggaaaaagaaaagtcaaaatagatattacaactgttggacgctctggatcaccaatacttcctccgatatctactcctcaaaattcaacaggtgggagaggaattattgctggaggcgtagaagccaaaattggcgcgtggccttggatggcagctgtttttgtgaaaaactttggcattggcagattccactgtgctggtagcataatcagtaacaagtacattttgtcagctgcccacgccttccttatcggaggtcgaaagttgaccccaactcgcttagctgtccgtgtgggaggccactacataaagaggggtcaagagtatccagtgaaagacgtgattatccatcctcattatgtagaaaaggagaactacaatgatatagccataatcgagttaaaagaggaactgaactttacggacttggtcaatcctatatgtctccctgatccagagacagtaacggatccattaaaagacagaattgtgactgcagcgggatggggcgatctggatttctccggtccacggagccaagttctacgtgaggtaagcatcccagttgttccagttgataaatgtgatcaagcctatgagaaactcaacaccccttcactaaaaaatgggataacgaataacttcctttgcgctggattggaagaaggagggaaagacgcttgccaaggcgattctggtggaccgttgatgctagtgaacaacactaggtggatagtagtaggagttgtgtcgttcgggcacaagtgtgccgaggaaggatatcctggtgtgtactcgcgcgtagcgagttacctagactggatcgcgaaagttacgaactcgttagatcatgccgtcactaactaa

SEQ ID NO: 6 - protein, 400 aa, Tachypleus tridentatus
MTWICVITLFALASATLGNKVSRVGVLFPKTRNDNECTARGGLKGSCKSLIDCPSVLATLKDSFPVVCSWNGRFQPIVCCPDAIAPPPVTTTAVTVISTKEPKLPRLHISGCGKRKVKIDITTVGRSGSPILPPISTPQNSTGGRGIIAGGVEAKIGAWPWMAAVFVKNFGIGRFHCAGSIISNKYILSAAHAFLIGGRKLTPTRLAVRVGGHYIKRGQEYPVKDVIIHPHYVEKENYNDIAIIELKEELNFTDLVNPICLPDPETVTDPLKDRIVTAAGWGDLDFSGPRSQVLREVSIPVVPVDKCDQAYEKLNTPSLKNGITNNFLCAGLEEGGKDACQGDSGGPLMLVNNTRWIVVGVVSFGHKCAEEGYPGVYSRVASYLDWIAKVTNSLDHAVTN

SEQ ID NO: 7 - DNA, 1128 bp, Tachypleus tridentatus
  source 1..1128: mol_type = genomic DNA
atgttggtgaataacgtgttttcactactgtgtttcccactcttgatgtctgtggttagatgcagtactctcagcagacagcgtagacagtttgttttccctgacgaggaagaactttgctcaaaccgatttactgaagaaggaacatgcaaaaatgtcttggattgtagaatacttttacaaaaaaatgattataatttactcaaagaatcaatatgcggctttgaaggcataacacccaaagtttgttgtccgaaatcaagccatgtaatttcaagtacacaggcacctccagaaaccactacgactgaacgcccaccaaaacagataccacccaatcttcatgaagtgtgtggaattcacaatactacaactaccaggattattggaggtcgggaagcacctattggagcctggccgtggatgactgctgtctacataaaacaaggaggaatcagaagtgttcagtgtggtggcgcacttgtcactaacaggcacgtgattacagcttcgcactgtgttgtaaacagtgcaggaacagatgtgatgccagctgatgtattctcggttcgtctgggtgaacacaatttatacagtaccgatgacgattcgaatccaatagattttgcagttacgtcggtgaaacatcacgaacactttgtactcgcgacgtatttgaatgacatcgcaattctaacgttaaatgacacagttacgtttacagacagaattcgacccatttgtctaccttatcgtaagttgagatacgatgatctagcaatgagaaaaccgtttatcactggatggggaacaacagcatttaacggcccatctagtgcagtgttgagagaagtacagttaccaatatgggaacacgaggcctgtagacaggcctacgagaaggatttaaatattacaaacgtgtatatgtgtgctggctttgcagatggcgggaaggatgcttgccagggtgattctggaggtccaatgatgttgcctgttaaaaccggagagttttatctcattggaattgtgtctttcggaaagaaatgcgcattgcctggatttcctggggtttacacaaaagtgacagagtttttagattggattgcagaacatatggtgtag

SEQ ID NO: 8 - protein, 375 aa, Tachypleus tridentatus
MLVNNVFSLLCFPLLMSVVRCSTLSRQRRQFVFPDEEELCSNRFTEEGTCKNVLDCRILLQKNDYNLLKESICGFEGITPKVCCPKSSHVISSTQAPPETTTTERPPKQIPPNLHEVCGIHNTTTTRIIGGREAPIGAWPWMTAVYIKQGGIRSVQCGGALVTNRHVITASHCVVNSAGTDVMPADVFSVRLGEHNLYSTDDDSNPIDFAVTSVKHHEHFVLATYLNDIAILTLNDTVTFTDRIRPICLPYRKLRYDDLAMRKPFITGWGTTAFNGPSSAVLREVQLPIWEHEACRQAYEKDLNITNVYMCAGFADGGKDACQGDSGGPMMLPVKTGEFYLIGIVSFGKKCALPGFPGVYTKVTEFLDWIAEHMV

SEQ ID NO: 9 - DNA, 1203 bp, Tachypleus tridentatus
  source 1..1203: mol_type = genomic DNA
atgacctggatctgcgtgatcaccctgttcgctctggcttccgctaccctgggcaacaaggtgtcccgtgtgggtgtcctgttccccaagacccgtaacgacaacgagtgcaccgctcgtggtggtctgaagggctcctgcaagtccctgatcgactgcccctccgtgctggctaccctgaaggactccttccccgtcgtgtgctcctggaacggtcgtttccagcccatcgtgtgctgccccgacgctatcgctcccccccctgtgaccaccaccgctgtgaccgtgatctccaccaaggagcccaagctgccccgtctgcacatctccggttgcggcaagcgcaaggtcaagatcgacatcaccaccgtgggccgttccggttcccccatcctgccccccatctccaccccccagaactccactggtggtcgtggtatcatcgctggcggtgtcgaggctaagatcggtgcttggccctggatggctgctgtgttcgtgaagaacttcggtatcggtcgcttccactgcgctggttccatcatctccaacaagtacatcctgtccgctgctcacgctttcctcatcggtggtcgcaagctgacccccacccgtctggctgtgcgtgtgggtggtcactacatcaagcgtggccaggagtaccccgtcaaggacgtgatcatccacccccactacgtggagaaggagaactacaacgacatcgccatcatcgagctgaaggaggagctgaacttcaccgacctggtcaaccccatctgcctgcccgaccccgagactgtgaccgaccctctgaaggaccgtatcgtgaccgctgctggctggggcgacctggacttctccggtccccgttcccaggtgctgcgtgaggtgtccatccccgtggtgcccgtggacaagtgcgaccaggcttacgagaagctgaacaccccctccctgaagaacggtattaccaacaacttcctctgcgccggactcgaggagggtggcaaggacgcttgccagggcgactccggtggtcccctgatgctggtcaacaacacccgttggatcgtcgtgggtgtcgtgtccttcggtcacaagtgcgctgaggagggttaccccggcgtctactcccgtgtggcttcctacctggactggatcgctaaggtcaccaactccctggaccacgctgtcaccaactaa

SEQ ID NO: 10 - protein, 4 aa, synthetic construct
IEGR